European Patent Application EP 4 317 176 A1, published February 7, 2024. Title: Vaccine composition based on attenuated reovirus and Use thereof. Applicant: Virocure Inc. The sequence listing filed with the application follows.

SEQUENCE LISTING (34 sequences)

SEQ ID NO: 1 - protein, 250 aa, Artificial Sequence
  RP116 sigma-1 protein
MDPRLREEVVRLIIALTSDNGVSLSKGLESRVSALEKTSQIHSDTILRITQGLDDANKRIIALEQSRDDLVASVSDAQLAISRLESSIGALQTVVNGLDSSVTQLGARVGQLETGLAELRVDHDNLVARVDTAERNIGSLTTELSTLTLRVTSIQADFESRISTLERTAVTSAGAPLSIRNNRMTMGLNDGLXLSGNNLAIRLPGNTGLNIQNGGLQFRFNTDQFQIVNNNLTLKTTVFDSINSRXGAXE

SEQ ID NO: 2 - DNA, 1416 bp, Artificial Sequence
  RP116 sigma-1 gene
gctattggtcggatggatcctcgcctacgtgaagaagtagtacggctgataatcgcattaacgagtgataatggagtatcactgtcaaaagggcttgaatcaagggtctcggcgctcgagaagacgtctcaaatacactctgatactatcctccggatcacccagggactcgatgatgcaaacaaacgaatcatcgctcttgagcaaagtcgggatgacttggttgcatcagtcagtgatgctcaacttgcaatctccagattggaaagctctatcggagccctccaaacagttgtcaatggacttgattcgagtgttacccagttgggtgctcgagtgggacaacttgagacaggacttgcagagctacgcgttgatcacgacaatctcgttgcgagagtggatactgcagaacgtaacattggatcattgaccactgagctatcaactctgacgttacgagtaacatccatacaagcggatttcgaatctaggatatccacattagagcgcacggcggtcactagcgcgggagctcccctctcaatccgtaataaccgtatgaccatgggattaaatgatggactcaygttgtcagggaataatctcgccatccgattgccaggaaatacgggtctgaatattcaaaatggtggacttcagtttcgatttaatactgatcaattccagatagttaataataacttgactctcaagacgactgtgtttgattctatcaactcaaggabaggcgcaaytgagtaaagtkmcgtggcgtcggcagtgactcccttgagattaaacagtagcacgaaggtgctggatatgctaatagacagttcaacacttgaaattaattctagtggacagctaactgttagatcgacatccccgaatttgaggtatccgatagctgatgttagcggcggtatcggaatgagtccaaattataggtttaggcagagcatgtggataggaattgtctcctattctggtagtgggctgaattggagggtacaggtgaactccgacatttttattgtagatgattacatacatatatgtcttccagcttttgacggtttctctatagctgacggtggagatctatcgttgaactttgttaccggattgttaccaccgttacttacaggagacactgagcccgcttttcataatgacgtggtcacatatggagcacagactgtagctatagggttgtcgtcgggtggtgcgcctcagtatatgagtaagaatctgtgggtggagcagtggcaggatggagtacttcggttacgtgttgaggggggtggctcaattacgcactcaaacagtaagtggcctgccatgaccgtttcgtacccgcgtagtttcacgtgaggatcagaccaccccgcggcactggggcatttcatc

SEQ ID NO: 3 - protein, 194 aa, Artificial Sequence
  RBD Amino Acid Sequence
NITNLCPFGEVFNATRFASVYAWNRKRISNCVADYSVLYNSASFSTFKCYGVSPTKLNDLCFTNVYADSFVIRGDEVRQIAPGQTGKIADYNYKLPDDFTGCVIAWNSNNLDSKVGGNYNYLYRLFRKSNLKPFERDISTEIYQAGSTPCNGVEGFNCYFPLQSYGFQPTNGVGYQPYRVVVLSFELLHAPATV

SEQ ID NO: 4 - protein, 8 aa, Artificial Sequence
  OVA257-264 Amino Acid Sequence
SIINFEKL

SEQ ID NO: 5 - protein, 17 aa, Artificial Sequence
  OVA323-339 Amino Acid Sequence
ISQAVHAAHAEINEAGR

SEQ ID NO: 6 - protein, 9 aa, Artificial Sequence
  Adpgk Amino Acid Sequence
ASMTNMELM

SEQ ID NO: 7 - protein, 8 aa, Artificial Sequence
  Rpl18 Amino Acid Sequence
KILTFDRL

SEQ ID NO: 8 - protein, 8 aa, Artificial Sequence
  P15E Amino Acid Sequence
KSPWFTTL

SEQ ID NO: 9 - protein, 18 aa, Artificial Sequence
  S21P2(1) Amino Acid Sequence
PSKPSKRSFIEDLLFNKV

SEQ ID NO: 10 - protein, 18 aa, Artificial Sequence
  S21P2(2) Amino Acid Sequence
PSKPSKRSFIEDLLFNKV

SEQ ID NO: 11 - protein, 5 aa, Artificial Sequence
  linker
GGGGS

SEQ ID NO: 12 - protein, 10 aa, Artificial Sequence
  c-Myc tag
EQKLISEEDL

SEQ ID NO: 13 - protein, 8 aa, Artificial Sequence
  FLAG tag
DYKDDDDK

SEQ ID NO: 14 - protein, 62 aa, Artificial Sequence
  OVA257-264 Construct Amino Acid Sequence
GGGGSGGGGSEQKLISEEDLSIINFEKLGGGGSSIINFEKLGGGGSSIINFEKLDYKDDDDK

SEQ ID NO: 15 - protein, 45 aa, Artificial Sequence
  OVA323-339 Construct Amino Acid Sequence
GGGGSGGGGSEQKLISEEDLISQAVHAAHAEINEAGRDYKDDDDK

SEQ ID NO: 16 - protein, 65 aa, Artificial Sequence
  Adpgk Construct Amino Acid Sequence
GGGGSGGGGSEQKLISEEDLASMTNMELMGGGGSASMTNMELMGGGGSASMTNMELMDYKDDDDK

SEQ ID NO: 17 - protein, 62 aa, Artificial Sequence
  Rpl18 Construct Amino Acid Sequence
GGGGSGGGGSEQKLISEEDLKILTFDRLGGGGSKILTFDRLGGGGSKILTFDRLDYKDDDDK

SEQ ID NO: 18 - protein, 62 aa, Artificial Sequence
  P15E Construct Amino Acid Sequence
GGGGSGGGGSEQKLISEEDLKSPWFTTLGGGGSKSPWFTTLGGGGSKSPWFTTLDYKDDDDK

SEQ ID NO: 19 - protein, 46 aa, Artificial Sequence
  S21P2(1) Construct Amino Acid Sequence
GGGGSGGGGSEQKLISEEDLPSKPSKRSFIEDLLFNKVDYKDDDDK

SEQ ID NO: 20 - protein, 69 aa, Artificial Sequence
  S21P2(2) Construct Amino Acid Sequence
GGGGSGGGGSEQKLISEEDLPSKPSKRSFIEDLLFNKVGGGGSPSKPSKRSFIEDLLFNKVDYKDDDDK

SEQ ID NO: 21 - DNA, 636 bp, Artificial Sequence
  RBD Codon Optimized Construct DNA Sequence
aatatcactaacttgtgtccgttcggcgaggtttttaatgcgaccaggtttgcttccgtgtacgcctggaacaggaaacggatctccaattgtgtcgccgattactccgtcttgtataattcagcatctttcagcacgtttaaatgttacggagtttcccccacaaaattgaatgacctttgctttacgaacgtctacgcggattcatttgtaatccggggggacgaagttaggcaaattgcgccagggcagactggcaagatagctgactataattataaattgccggatgactttacgggctgtgtgattgcttggaactcaaataatctggactcaaaggtagggggaaattataactacctttacaggctgttccggaagagtaatctgaagccattcgaaagagatataagtacagagatctaccaagctggaagcaccccctgcaatggtgttgaaggattcaattgttatttcccattgcaatcctatggttttcaaccgacgaatggggtgggataccaaccatatcgagttgtggttctcagtttcgagttgcttcatgctcctgcgacagtatgtggaccaaaaaaatctactaatctggtgaagaataaatgcgtcaatttttaa

SEQ ID NO: 22 - DNA, 189 bp, Artificial Sequence
  OVA257-264 Codon Optimized Construct DNA Sequence
ggaggtggaggctcaggtggcggaggttctgagcagaagttgatttcagaggaagatctgagtattataaacttcgagaagctgggtgggggaggaagttcaatcattaattttgaaaaacttggaggaggtggatcttccataattaattttgaaaagctggattataaggatgacgacgataagtga

SEQ ID NO: 23 - DNA, 138 bp, Artificial Sequence
  OVA323-339 Codon Optimized Construct DNA Sequence
ggaggtggaggctcaggtggcggaggttctgagcagaagttgatttcagaggaagatctgatttcacaggctgtgcatgctgcacatgctgaaattaatgaggctggacgtgattataaggatgacgacgataagtga

SEQ ID NO: 24 - DNA, 198 bp, Artificial Sequence
  Adpgk Codon Optimized Construct DNA Sequence
ggaggtggaggctcaggtggcggaggttctgagcagaagttgatttcagaggaagatctggctagcatgacgaacatggagctaatgggagggggcggaagtgcttctatgactaatatggaactgatgggaggtggaggttctgcttcaatgaccaacatggaacttatggattataaggatgacgacgataagtga

SEQ ID NO: 25 - DNA, 189 bp, Artificial Sequence
  Rpl18 Codon Optimized Construct DNA Sequence
ggaggtggaggctcaggtggcggaggttctgagcagaagttgatttcagaggaagatctgaagattctgacgtttgatcgtctggggggtggcggatctaagatattgacgttcgatcgactgggaggaggtggctctaagatcctaacattcgaccgtctagattataaggatgacgacgataagtga

SEQ ID NO: 26 - DNA, 189 bp, Artificial Sequence
  P15E Codon Optimized Construct DNA Sequence
ggaggtggaggctcaggtggcggaggttctgagcagaagttgatttcagaggaagatctgaagtcaccttggtttactactctcggtgggggaggaagtaaatcgccatggtttactacattgggaggaggtgggtctaagtcaccatggttcacgacattggattataaggatgacgacgataagtga

SEQ ID NO: 27 - DNA, 141 bp, Artificial Sequence
  S21P2(1) Codon Optimized Construct DNA Sequence
ggaggtggaggctcaggtggcggaggttctgagcagaagttgatttcagaggaagatctgcctagtaagccttctaagcgcagcttcatagaagatttgttgttcaataaggtagattataaggatgacgacgataagtga

SEQ ID NO: 28 - DNA, 210 bp, Artificial Sequence
  S21P2(2) Codon Optimized Construct DNA Sequence
ggaggtggaggctcaggtggcggaggttctgagcagaagttgatttcagaggaagatctgcctagtaagccttctaagcgcagcttcatagaagatttgttgttcaataaggtaggtgggggaggaagtccatcgaagccaagtaagcgtagtttcattgaggacctcctcttcaacaaggttgattataaggatgacgacgataagtga

SEQ ID NO: 29 - DNA, 20 bp, Artificial Sequence
  S1 fwd
cacccagggactcgatgatg

SEQ ID NO: 30 - DNA, 20 bp, Artificial Sequence
  S1 rev
gcacccaactgggtaacact

SEQ ID NO: 31 - DNA, 40 bp, Artificial Sequence
  RBD fwd
caactgagcaaagttacgtgagggtacaacctacggaatc

SEQ ID NO: 32 - DNA, 61 bp, Artificial Sequence
  RBD rev
atgaaatgccccagtgccgcggggtggtctgacctcaaaaattgacgcatttattcttcac

SEQ ID NO: 33 - DNA, 39 bp, Artificial Sequence
  S1-250-AvrII-F
gattctatcaactcaaggataggcgcaattgagcctagg

SEQ ID NO: 34 - DNA, 45 bp, Artificial Sequence
  pBacT7-SacII-R
cagtgccgcggggtggtctgatcctcacgtgaaactacgcgggta